European Patent Application EP 4 375 382 A2, published May 29, 2024. Title: BACTERIAL STRAINS HAVING FUNGICIDAL ACTIVITY, COMPOSITIONS COMPRISING SAME AND USE THEREOF. Applicant: Lavie Bio Ltd. Application EP. The sequence listing filed with the application follows.

SEQUENCE LISTING (76 sequences)

SEQ ID NO: 1 - DNA, 1407 bp, Serratia sp.
  misc_feature 1..1407: note = ribosomal RNA nucleic acid sequence
  source 1..1407: mol_type = genomic DNA
tcatggctcagattgaacgctggcggcaggcctaacacatgcaagtcgagcggtagcacaggagagcttgctctctgggtgacgagcggcggacgggtgagtaatgtctgggaaactgcctgatggagggggataactactggaaacggtagctaataccgcataacgtctacggaccaaagtgggggaccttcgggcctcacgccatcagatgtgcccagatgggattagctagtaggtggggtaatggctcacctaggcgacgatccctagctggtctgagaggatgaccagccacactggaactgagacacggtccagactcctacgggaggcagcagtggggaatattgcacaatgggcgcaagcctgatgcagccatgccgcgtgtgtgaagaaggccttagggttgtaaagcactttcagcgaggaggaagggtagtgtgttaatagcacattgcattgacgttactcgcagaagaagcaccggctaactccgtgccagcagccgcggtaatacggagggtgcaagcgttaatcggaattactgggcgtaaagcgcacgcaggcggtttgttaagtcagatgtgaaatccccgcgcttaacgtgggaactgcatttgaaactggcaagctagagtcttgtagaggggggtagaattccaggtgtagcggtgaaatgcgtagagatctggaggaataccggtggcgaaggcggccccctggacaaagactgacgctcaggtgcgaaagcgtggggagcaaacaggattagataccctggtagtccacgctgtaaacgatgtcgatttggaggttgtgcccttgaggcgtggcttccggagctaacgcgttaaatcgaccgcctggggagtacggccgcaaggttaaaactcaaatgaattgacgggggcccgcacaagcggtggagcatgtggtttaattcgatgcaacgcgaagaaccttacctactcttgacatccagagaactttccagagatggattggtgccttcgggaactctgagacaggtgctgcatggctgtcgtcagctcgtgttgtgaaatgttgggttaagtcccgcaacgagcgcaacccttatcctttgttgccagcgattcggtcgggaactcaaaggagactgccggtgataaaccggaggaaggtggggatgacgtcaagtcatcatggcccttacgagtagggctacacacgtgctacaatggcgtatacaaagagaagcgaactcgcgagagcaagcggacctcataaagtacgtcgtagtccggattggagtctgcaactcgactccatgaagtcggaatcgctagtaatcgtagatcagaatgctacggtgaatacgttcccgggccttgtacacaccgcccgtcacaccatgggagtggg

SEQ ID NO: 2 - DNA, 1520 bp, Pseudomonas sp.
  misc_feature 1..1520: note = ribosomal RNA nucleic acid sequence
  source 1..1520: mol_type = genomic DNA
aagagtttgatcatggctcagattgaacgctggcggcaggcctaacacatgcaagtcgagcggtagagagaagcttgcttctcttgagagcggcggacgggtgagtaatgcctaggaatctgcctggtagtgggggataacgtccggaaacggacgctaataccgcatacgtcctacgggagaaagcaggggaccttcgggccttgcgctatcagatgagcctaggtcggattagctagttggtgaggtaatggctcaccaaggcgacgatccgtaactggtctgagaggatgatcagtcacactggaactgagacacggtccagactcctacgggaggcagcagtggggaatattggacaatgggcgaaagcctgatccagccatgccgcgtgtgtgaagaaggtcttcggattgtaaagcactttaagttgggaggaagggtacttacctaatacgtgagtattttgacgttaccgacagaataagcaccggctaactctgtgccagcagccgcggtaatacagagggtgcaagcgttaatcggaattactgggcgtaaagcgcgcgtaggtggttcgttaagttggatgtgaaatccccgggctcaacctgggaactgcatccaaaactggcgagctagagtatggtagagggtggtggaatttcctgtgtagcggtgaaatgcgtagatataggaaggaacaccagtggcgaaggcgaccacctggactgatactgacactgaggtgcgaaagcgtggggagcaaacaggattagataccctggtagtccacgccgtaaacgatgtcaactagccgttgggagccttgagctcttagtggcgcagctaacgcattaagttgaccgcctggggagtacggccgcaaggttaaaactcaaatgaattgacgggggcccgcacaagcggtggagcatgtggtttaattcgaagcaacgcgaagaaccttaccaggccttgacatccaatgaactttccagagatggattggtgccttcgggaacattgagacaggtgctgcatggctgtcgtcagctcgtgtcgtgagatgttgggttaagtcccgtaacgagcgcaacccttgtccttagttaccagcacgttatggtgggcactctaaggagactgccggtgacaaaccggaggaaggtggggatgacgtcaagtcatcatggcccttacggcctgggctacacacgtgctacaatggtcggtacagagggttgccaagccgcgaggtggagctaatcccataaaaccgatcgtagtccggatcgcagtctgcaactcgactgcgtgaagtcggaatcgctagtaatcgcgaatcagaatgtcgcggtgaatacgttcccgggccttgtacacaccgcccgtcacaccatgggagtgggttgcaccagaagtagctagtctaaccttcgggaggacggttaccacggtgtgattcatgactggggtgaagtcgtaacaaggtagccgtaggggaacctgcggctgga

SEQ ID NO: 3 - DNA, 1396 bp, Pseudomonas sp.
  misc_feature 1..1396: note = ribosomal RNA nucleic acid sequence
  source 1..1396: mol_type = genomic DNA
cccactcccatggtgtgacgggcggtgtgtacaaggcccgggaacgtattcaccgcgacattctgattcgcgattactagcgattccgacttcacgcagtcgagttgcagactgcgatccggactacgatcggttttatgggattagctccacctcgcggcttggcaaccctctgtaccgaccattgtagcacgtgtgtagcccaggccgtaagggccatgatgacttgacgtcatccccaccttcctccggtttgtcaccggcagtctccttagagtgcccaccataacgtgctggtaactaaggacaagggttgcgctcgttacgggacttaacccaacatctcacgacacgagctgacgacagccatgcagcacctgtctcaatgttcccgaaggcaccaatccatctctggaaagttcattggatgtcaaggcctggtaaggttcttcgcgttgcttcgaattaaaccacatgctccaccgcttgtgcgggcccccgtcaattcatttgagttttaaccttgcggccgtactccccaggcggtcaacttaatgcgttagctgcgccactaagagctcaaggctcccaacggctagttgacatcgtttacggcgtggactaccagggtatctaatcctgtttgctccccacgctttcgcacctcagtgtcagtatcagtccaggtggtcgccttcgccactggtgttccttcctatatctacgcatttcaccgctacacaggaaattccaccaccctctaccatactctagctcgccagttttggatgcagttcccaggttgagcccggggatttcacatccaacttaacgaaccacctacgcgcgctttacgcccagtaattccgattaacgcttgcaccctctgtattaccgcggctgctggcacagagttagccggtgcttattctgtcggtaacgtcaaaatactcacgtattaggtaagtacccttcctcccaacttaaagtgctttacaatccgaagaccttcttcacacacgcggcatggctggatcaggctttcgcccattgtccaatattccccactgctgcctcccgtaggagtctggaccgtgtctcagttccagtgtgactgatcatcctctcagaccagttacggatcgtcgccttggtgagccattacctcaccaactagctaatccgacctaggctcatctgatagcgcaaggcccgaaggtcccctgctttctcccgtaggacgtatgcggtattagcgtccgtttccggacgttatcccccactaccaggcagattcctaggcattactcacccgtccgccgctctcaagagaagcaagcttctctctaccgctcgacttgcatgtgttaggcctgccgccagcgttcaatctgag

SEQ ID NO: 4 - DNA, 1430 bp, Streptomyces sp.
  misc_feature 1..1430: note = ribosomal RNA nucleic acid sequence
  source 1..1430: mol_type = genomic DNA
tggctcaggacgaacgctggcggcgtgcttaacacatgcaagtcgaacgatgaagcctttcggggtggattagtggcgaacgggtgagtaacacgtgggcaatctgcccttcactctgggacaagccctggaaacggggtctaataccggataacactctgtcctgcatgggacggggttaaaagctccggcggtgaaggatgagcccgcggcctatcagcttgttggtggggtaatggcctaccaaggcgacgacgggtagccggcctgagagggcgaccggccacactgggactgagacacggcccagactcctacgggaggcagcagtggggaatattgcacaatgggcgaaagcctgatgcagcgacgccgcgtgagggatgacggccttcgggttgtaaacctctttcagcagggaagaagcgaaagtgacggtacctgcagaagaagcgccggctaactacgtgccagcagccgcggtaatacgtagggcgcaagcgttgtccggaattattgggcgtaaagagctcgtaggcggcttgtcacgtcggatgtgaaagcccggggcttaaccccgggtctgcattcgatacgggctagctagagtgtggtaggggagatcggaattcctggtgtagcggtgaaatgcgcagatatcaggaggaacaccggtggcgaaggcggatctctgggccattactgacgctgaggagcgaaagcgtggggagcgaacaggattagataccctggtagtccacgccgtaaacgttgggaactaggtgttggcgacattccacgtcgtcggtgccgcagctaacgcattaagttccccgcctggggagtacggccgcaaggctaaaactcaaaggaattgacgggggcccgcacaagcagcggagcatgtggcttaattcgacgcaacgcgaagaaccttaccaaggcttgacatataccggaaagcatcagagatggtgccccccttgtggtcggtatacaggtggtgcatggctgtcgtcagctcgtgtcgtgagatgttgggttaagtcccgcaacgagcgcaacccttgttctgtgttgccagcatgcccttcggggtgatggggactcacaggagactgccggggtcaactcggaggaaggtggggacgacgtcaagtcatcatgccccttatgtcttgggctgcacacgtgctacaatggccggtacaatgagctgcgatgccgcgaggcggagcgaatctcaaaaagccggtctcagttcggattggggtctgcaactcgaccccatgaagtcggagttgctagtaatcgcagatcagcattgctgcggtgaatacgttcccgggccttgtacacaccgcccgtcacgtcacgaaagtcggtaacacccgaagccggtggcccaaccccttgtgggagggagctgt

SEQ ID NO: 5 - DNA, 1417 bp, Pseudomonas sp.
  misc_feature 1..1417: note = ribosomal RNA nucleic acid sequence
  source 1..1417: mol_type = genomic DNA
agactagctacttctggtgcaacccactcccatggtgtgacgggcggtgtgtacaaggcccgggaacgtattcaccgcgacattctgattcgcgattactagcgattccgacttcacgcagtcgagttgcagactgcgatccggactacgatcggttttgtgggattagctccacctcgcggcttggcaaccctctgtaccgaccattgtagcacgtgtgtagcccaggccgtaagggccatgatgacttgacgtcatccccaccttcctccggtttgtcaccggcagtctccttagagtgcccaccataacgtgctggtaactaaggacaagggttgcgctcgttacgggacttaacccaacatctcacgacacgagctgacgacagccatgcagcacctgtctcaatgttcccgaaggcaccaatccatctctggaaagttcattggatgtcaaggcctggtaaggttcttcgcgttgcttcgaattaaaccacatgctccaccgcttgtgcgggcccccgtcaattcatttgagttttaaccttgcggccgtactccccaggcggtcaacttaatgcgttagctgcgccactaagagctcaaggctcccaacggctagttgacatcgtttacggcgtggactaccagggtatctaatcctgtttgctccccacgctttcgcacctcagtgtcagtatcagtccaggtggtcgccttcgccactggtgttccttcctatatctacgcatttcaccgctacacaggaaattccaccaccctctaccatactctagctcgacagttttgaatgcagttcccaggttgagcccggggatttcacatccaacttaacgaaccacctacgcgcgctttacgcccagtaattccgattaacgcttgcaccctctgtattaccgcggctgctggcacagagttagccggtgcttattctgtcggtaacgtcaaaacactaacgtattaggttaatgcccttcctcccaacttaaagtgctttacaatccgaagaccttcttcacacacgcggcatggctggatcaggctttcgcccattgtccaatattccccactgctgcctcccgtaggagtctggaccgtgtctcagttccagtgtgactgatcatcctctcagaccagttacggatcgtcgccttggtgagccattaccccaccaactagctaatccgacctaggctcatctgatagcgcaaggcccgaaggtcccctgctttctcccgtaggacgtatgcggtattagcgtccgtttccgagcgttatcccccactaccaggcagattcctaggcattactcacccgtccgccgctctcaagaggtgcaagcacctctctaccgctcgacttgcatgtgttaggcctgccgccagcgttcaatctga

SEQ ID NO: 6 - DNA, 1465 bp, Pseudomonas sp.
  misc_feature 1..1465: note = ribosomal RNA nucleic acid sequence
  source 1..1465: mol_type = genomic DNA
cagtcatgaatcacaccgtggtaaccgtccccccgaaggttagactagctacttctggtgcaacccactcccatggtgtgacgggcggtgtgtacaaggcccgggaacgtattcaccgcgacattctgattcgcgattactagcgattccgacttcacgcagtcgagttgcagactgcgatccggactacgatcggttttgtgggattagctccacctcgcggcttggcaaccctctgtaccgaccattgtagcacgtgtgtagcccaggccgtaagggccatgatgacttgacgtcatccccaccttcctccggtttgtcaccggcagtctccttagagtgcccaccataacgtgctggtaactaaggacaagggttgcgctcgttacgggacttaacccaacatctcacgacacgagctgacgacagccatgcagcacctgtctcaatgttcccgaaggcaccaatccatctctggaaagttcattggatgtcaaggcctggtaaggttcttcgcgttgcttcgaattaaaccacatgctccaccgcttgtgcgggcccccgtcaattcatttgagttttaaccttgcggccgtactccccaggcggtcaacttaatgcgttagctgcgccactaagagctcaaggctcccaacggctagttgacatcgtttacggcgtggactaccagggtatctaatcctgtttgctccccacgctttcgcacctcagtgtcagtatcagtccaggtggtcgccttcgccactggtgttccttcctatatctacgcatttcaccgctacacaggaaattccaccaccctctaccatactctagctcgacagttttgaatgcagttcccaggttgagcccggggatttcacatccaacttaacgaaccacctacgcgcgctttacgcccagtaattccgattaacgcttgcaccctctgtattaccgcggctgctggcacagagttagccggtgcttattctgtcggtaacgtcaaaacactaacgtattaggttaatgcccttcctcccaacttaaagtgctttacaatccgaagaccttcttcacacacgcggcatggctggatcaggctttcgcccattgtccaatattccccactgctgcctcccgtaggagtctggaccgtgtctcagttccagtgtgactgatcatcctctcagaccagttacggatcgtcgccttggtgagccattaccccaccaactagctaatccgacctaggctcatctgatagcgcaaggcccgaaggtcccctgctttctcccgtaggacgtatgcggtattagcgtccgtttccgagcgttatcccccactaccaggcagattcctaggcattactcacccgtccgccgctctcaagaggtgcaagcacctctctaccgctcgacttgcatgtgttaggcctgccgccagcgttcaatctgagccatga

SEQ ID NO: 7 - DNA, 1468 bp, Pantoea sp.
  misc_feature 439: note = n is a, c, g, or t
  misc_feature 441: note = n is a, c, g, or t
  misc_feature 453: note = n is a, c, g, or t
  misc_feature 982..983: note = n is a, c, g, or t
  misc_feature 987: note = n is a, c, g, or t
  misc_feature 990: note = n is a, c, g, or t
  misc_feature 1001: note = n is a, c, g, or t
  misc_feature 1004: note = n is a, c, g, or t
  misc_feature 1019..1020: note = n is a, c, g, or t
  misc_feature 1..1468: note = ribosomal RNA nucleic acid sequence
  source 1..1468: mol_type = genomic DNA
catggctcagattgaacgctggcggcaggcctaacacatgcaagtcggacggtagcacagagagcttgctcttgggtgacgagtggcggacgggtgagtaatgtctggggatctgcccgatagagggggataaccactggaaacggtggctaataccgcataacgtcgcaagaccaaagagggggaccttcgggcctctcactatcggatgaacccagatgggattagctagtaggcggggtaatggcccacctaggcgacgatccctagctggtctgagaggatgaccagccacactggaactgagacacggtccagactcctacgggaggcagcagtggggaatattgcacaatgggcgcaagcctgatgcagccatgccgcgtgtatgaagaaggccttcgggttgtaaagtactttcagcggggaggaaggcgangnggttaataaccntgtcgattgacgttacccgcagaagaagcaccggctaactccgtgccagcagccgcggtaatacggagggtgcaagcgttaatcggaattactgggcgtaaagcgcacgcaggcggtctgttaagtcagatgtgaaatccccgggcttaacctgggaactgcatttgaaactggcaggcttgagtcttgtagaggggggtagaattccaggtgtagcggtgaaatgcgtagagatctggaggaataccggtggcgaaggcggccccctggacaaagactgacgctcaggtgcgaaagcgtggggagcaaacaggattagataccctggtagtccacgccgtaaacgatgtcgacttggaggttgttcccttgaggagtggcttccggagctaacgcgttaagtcgaccgcctggggagtacggccgcaaggttaaaactcaaatgaattgacgggggcccgcacaagcggtggagcatgtggtttaattcgatgcaacgcgaagaaccttacctactcttgacatccanngaanttngcagagatgcnttngtgccttcgggaacnntgagacaggtgctgcatggctgtcgtcagctcgtgttgtgaaatgttgggttaagtcccgcaacgagcgcaacccttatcctttgttgccagcgattcggtcgggaactcaaaggagactgccggtgataaaccggaggaaggtggggatgacgtcaagtcatcatggcccttacgagtagggctacacacgtgctacaatggcgcatacaaagagaagcgacctcgcgagagcaagcggacctcacaaagtgcgtcgtagtccggatcggagtctgcaactcgactccgtgaagtcggaatcgctagtaatcgtggatcagaatgccacggtgaatacgttcccgggccttgtacacaccgcccgtcacaccatgggagtgggttgcaaaagaagtaggtagcttaaccttcgggagggcgcttaccactttgtgattcatgactgg

SEQ ID NO: 8 - DNA, 1522 bp, Enterobacter sp.
  misc_feature 1..1522: note = ribosomal RNA nucleic acid sequence
  source 1..1522: mol_type = genomic DNA
agagtttgatcatggctcagattgaacgctggcggcaggcctaacacatgcaagtcgaacggtagcacagagagcttgctctcgggtgacgagtggcggacgggtgagtaatgtctgggaaactgcctgatggagggggataactactggaaacggtagctaataccgcataacgtcgcaagaccaaagagggggaccttcgggcctcttgccatcagatgtgcccagatgggattagctagtaggtggggtaacggctcacctaggcgacgatccctagctggtctgagaggatgaccagccacactggaactgagacacggtccagactcctacgggaggcagcagtggggaatattgcacaatgggcgcaagcctgatgcagccatgccgcgtgtatgaagaaggccttcgggttgtaaagtactttcagcggggaggaaggtgttgtggttaataaccacagcaattgacgttacccgcagaagaagcaccggctaactccgtgccagcagccgcggtaatacggagggtgcaagcgttaatcggaattactgggcgtaaagcgcacgcaggcggtctgtcaagtcggatgtgaaatccccgggctcaacctgggaactgcattcgaaactggcaggctagagtcttgtagaggggggtagaattccaggtgtagcggtgaaatgcgtagagatctggaggaataccggtggcgaaggcggccccctggacaaagactgacgctcaggtgcgaaagcgtggggagcaaacaggattagataccctggtagtccacgccgtaaacgatgtcgacttggaggttgtgcccttgaggcgtggcttccggagctaacgcgttaagtcgaccgcctggggagtacggccgcaaggttaaaactcaaatgaattgacgggggcccgcacaagcggtggagcatgtggtttaattcgatgcaacgcgaagaaccttacctactcttgacatccagagaactttccagagatggattggtgccttcgggaactctgagacaggtgctgcatggctgtcgtcagctcgtgttgtgaaatgttgggttaagtcccgcaacgagcgcaacccttatcctttgttgccagcggtccggccgggaactcaaaggagactgccagtgataaactggaggaaggtggggatgacgtcaagtcatcatggcccttacgagtagggctacacacgtgctacaatggcgcatacaaagagaagcgaactcgcgagagcaagcggacctcataaagtgcgtcgtagtccggattggagtctgcaactcgactccatgaagtcggaatcgctagtaatcgtagatcagaatgctacggtgaatacgttcccgggccttgtacacaccgcccgtcacaccatgggagtgggttgcaaaagaagtaggtagcttaaccttcgggagggcgcttaccactttgtgattcatgactggggtgaagtcgtaacaaggtaaccgtaggggaacctgcggttgga

SEQ ID NO: 9 - DNA, 1330 bp, Enterobacter sp.
  misc_feature 50: note = n is a, c, g, or t
  misc_feature 57: note = n is a, c, g, or t
  misc_feature 108: note = n is a, c, g, or t
  misc_feature 115: note = n is a, c, g, or t
  misc_feature 172: note = n is a, c, g, or t
  misc_feature 176: note = n is a, c, g, or t
  misc_feature 178: note = n is a, c, g, or t
  misc_feature 323: note = n is a, c, g, or t
  misc_feature 335: note = n is a, c, g, or t
  misc_feature 1..1330: note = ribosomal RNA nucleic acid sequence
  source 1..1330: mol_type = genomic DNA
atggagggggataactactggaaacggtagctaataccgcataacgtcgnaagaccnaagagggggaccttcgggcgctcttgccatcagatgtgcccagatgggatnagctagnaggtggggtaacggctcacctaggcgacgatccctagctggtctgagaggatgaccngccncnctggaactgagacacggtccagactcctacgggaggcagcagtggggaatattgcacaatgggcgcaagcctgatgcagccatgccgcgtgtatgaagaaggccttcgggttgtaaagtactttcagcggggaggaaggtgttgnggttaataaccncagcaattgacgttacccgcagaagaagcaccggctaactccgtgccagcagccgcggtaatacggagggtgcaagcgttaatcggaattactgggcgtaaagcgcacgcaggcggtctgtcaagtcggatgtgaaatccccgggctcaacctgggaactgcattcgaaactggcaggctagagtcttgtagaggggggtagaattccaggtgtagcggtgaaatgcgtagagatctggaggaataccggtggcgaaggcggccccctggacaaagactgacgctcaggtgcgaaagcgtggggagcaaacaggattagataccctggtagtccacgccgtaaacgatgtcgacttggaggttgtgcccttgaggcgtggcttccggagctaacgcgttaagtcgaccgcctggggagtacggccgcaaggttaaaactcaaatgaattgacgggggcccgcacaagcggtggagcatgtggtttaattcgatgcaacgcgaagaaccttacctactcttgacatccagagaactttccagagatggattggtgccttcgggaactctgagacaggtgctgcatggctgtcgtcagctcgtgttgtgaaatgttgggttaagtcccgcaacgagcgcaacccttatcctttgttgccagcggtccggccgggaactcaaaggagactgccagtgataaactggaggaaggtggggatgacgtcaagtcatcatggcccttacgagtagggctacacacgtgctacaatggcgcatacaaagagaagcgaactcgcgagagcaagcggacctcataaagtgcgtcgtagtccggattggagtctgcaactcgactccatgaagtcggaatcgctagtaatcgtagatcagaatgctacggtgaatacgttcccgggccttgtacacaccgcccgtcacaccatgggagtgggttgcaaaagaagtaggtagcttaaccttcgggagggcgcttacc

SEQ ID NO: 10 - DNA, 1480 bp, Pseudomonas sp.
  misc_feature 365: note = n is a, c, g, or t
  misc_feature 1..1480: note = ribosomal RNA nucleic acid sequence
  source 1..1480: mol_type = genomic DNA
ctgtacgacttcaccccagtcatgaatcacaccgtggtaaccgtcctcccgaaggttagactagctacttctggtgcaacccactcccatggtgtgacgggcggtgtgtacaaggcccgggaacgtattcaccgcgacattctgattcgcgattactagcgattccgacttcacgcagtcgagttgcagactgcgatccggactacgatcggttttgtgagattagctccacctcgcggcttggcaaccctctgtaccgaccattgtagcacgtgtgtagcccaggccgtaagggccatgatgacttgacgtcatccccaccttcctccggtttgtcaccggcagtctccttagagtgcccaccntaacgtgctggtaactaaggacaagggttgcgctcgttacgggacttaacccaacatctcacgacacgagctgacgacagccatgcagcacctgtctcaatgttcccgaaggcaccaatccatctctggaaagttcattggatgtcaaggcctggtaaggttcttcgcgttgcttcgaattaaaccacatgctccaccgcttgtgcgggcccccgtcaattcatttgagttttaaccttgcggccgtactccccaggcggtcaacttaatgcgttagctgcgccactaagagttcaagactcccaacggctagttgacatcgtttacggcgtggactaccagggtatctaatcctgtttgctccccacgctttcgcacctcagtgtcagtatgagcccaggtggtcgccttcgccactggtgttccttcctatatctacgcatttcaccgctacacaggaaattccaccaccctctgccctactctagcttgccagttttggatgcagttcccaggttgagcccggggatttcacattcaacttaacaaaccacctacgcgcgctttacgcccagtaattccgattaacgcttgcaccctctgtattaccgcggctgctggcacagagttagccggtgcttattctgtcggtaacgtcaagacagcaaggtattcgctgactgcccttcctcccaacttaaagtgctttacaatccgaagaccttcttcacacacgcggcatggctggatcaggctttcgcccattgtccaatattccccactgctgcctcccgtaggagtctggaccgtgtctcagttccagtgtgactgatcatcctctcagaccagttacggatcgtcgccttggtgagccattacctcaccaactagctaatccgacctaggctcatctgatagcgcaaggcccgaaggtcccctgctttctcccgtaggacgtatgcggtattagcgttcctttcgaaacgttgtcccccactaccaggcagattcctaggcattactcacccgtccgccgctgaatcaggaagcaagcttccttcaaccgctcgacttgcatgtgttaggcctgccgccagcgttcaatctgagccatg

SEQ ID NO: 11 - DNA, 1488 bp, Erwinia sp.
  misc_feature 497: note = n is a, c, g, or t
  misc_feature 1036: note = n is a, c, g, or t
  misc_feature 1038: note = n is a, c, g, or t
  misc_feature 1047: note = n is a, c, g, or t
  misc_feature 1413: note = n is a, c, g, or t
  misc_feature 1..1488: note = ribosomal RNA nucleic acid sequence
  source 1..1488: mol_type = genomic DNA
cctgttacgacttcaccccagtcatgaatcacaaagtggtaagcgccctcccgaaggttaagctacctacttcttttgcaacccactcccatggtgtgacgggcggtgtgtacaaggcccgggaacgtattcaccgtggcattctgatccacgattactagcgattccgacttcacggagtcgagttgcagactccgatccggactacgacgcactttgtgaggtccgcttgctctcgcgaggtcgcttctctttgtatgcgccattgtagcacgtgtgtagccctgctcgtaagggccatgatgacttgacgtcatccccaccttcctccggtttatcaccggcagtctcctttgagttcccgaccgaatcgctggcaacaaaggataagggttgcgctcgttgcgggacttaacccaacatttcacaacacgagctgacgacagccatgcagcacctgtctcacggttcccgaaggcactaaggcatctctgccnaattccgtggatgtcaagagcaggtaaggttcttcgcgttgcatcgaattaaaccacatgctccaccgcttgtgcgggcccccgtcaattcatttgagttttaaccttgcggccgtactccccaggcggtcgacttaacgcgttagctccggaagccacgagtcatgctcacagcctccaagtcgacatcgtttacggcgtggactaccagggtatctaatcctgtttgctccccacgctttcgcacctgagcgtcagtctttgtccagggggccgccttcgccaccggtattcctccagatctctacgcatttcaccgctacacctggaattctacccccctctacaagactcaagcctgccagtttcaaatgcagttcccaggttaagcccggggatttcacatctgacttaacagaccgcctgcgtgcgctttacgcccagtaattccgattaacgcttgcaccctccgtattaccgcggctgctggcacggagttagccggtgcttcttctgcgggtaacgtcaatgaacgaggntnttaacctcntccccttcctccccgctgaaagtactttacaacccgaaggccttcttcatacacgcggcatggctgcatcaggcttgcgcccattgtgcaatattccccactgctgcctcccgtaggagtctggaccgtgtctcagttccagtgtggctggtcatcctctcagaccagctagggatcgtcgcctaggtgagccgttaccccacctactagctaatcccatctgggttcatccgatggtgtgaggcccgaaggtcccccactttggtcttgcgacgttatgcggtattagccaccgtttccagtggttatccccctccatcgggcagatccccagacattactcacccgtccgccactcgtcacccnaggagcaagctcctctgtgctaccgttcgacttgcatgtgttaggcctgccgccagcgttcaatctgagccatga

SEQ ID NO: 12 - DNA, 1425 bp, Pantoea sp.
  misc_feature 369: note = n is a, c, g, or t
  misc_feature 920..921: note = n is a, c, g, or t
  misc_feature 930..931: note = n is a, c, g, or t
  misc_feature 1..1425: note = ribosomal RNA nucleic acid sequence
  source 1..1425: mol_type = genomic DNA
cttgggtgacgagtggcggacgggtgagtaatgtctggggatctgcccgatagagggggataaccactggaaacggtggctaataccgcataacgtcgcaagaccaaagagggggaccttcgggcctctcactatcggatgaacccagatgggattagctagtaggcggggtaatggcccacctaggcgacgatccctagctggtctgagaggatgaccagccacactggaactgagacacggtccagactcctacgggaggcagcagtggggaatattgcacaatgggcgcaagcctgatgcagccatgccgcgtgtatgaagaaggccttcgggttgtaaagtactttcagcggggaggaaggcganggggttaataaccctgtcgattgacgttacccgcagaagaagcaccggctaactccgtgccagcagccgcggtaatacggagggtgcaagcgttaatcggaattactgggcgtaaagcgcacgcaggcggtctgttaagtcagatgtgaaatccccgggcttaacctgggaactgcatttgaaactggcaggcttgagtcttgtagaggggggtagaattccaggtgtagcggtgaaatgcgtagagatctggaggaataccggtggcgaaggcggccccctggacaaagactgacgctcaggtgcgaaagcgtggggagcaaacaggattagataccctggtagtccacgccgtaaacgatgtcgacttggaggttgttcccttgaggagtggcttccggagctaacgcgttaagtcgaccgcctggggagtacggccgcaaggttaaaactcaaatgaattgacgggggcccgcacaagcggtggagcatgtggtttaattcgatgcaacgcgaagaaccttacctactcttgacatccagcgaacttnncagagatgnnttggtgccttcgggaacgctgagacaggtgctgcatggctgtcgtcagctcgtgttgtgaaatgttgggttaagtcccgcaacgagcgcaacccttatcctttgttgccagcgattcggtcgggaactcaaaggagactgccggtgataaaccggaggaaggtggggatgacgtcaagtcatcatggcccttacgagtagggctacacacgtgctacaatggcgcatacaaagagaagcgacctcgcgagagcaagcggacctcacaaagtgcgtcgtagtccggatcggagtctgcaactcgactccgtgaagtcggaatcgctagtaatcgtggatcagaatgccacggtgaatacgttcccgggccttgtacacaccgcccgtcacaccatgggagtgggttgcaaaagaagtaggtagcttaaccttcgggagggcgcttaccactttgtgattcatgactggggtgaagtcgtaacagggtaaccgtaa

SEQ ID NO: 13 - DNA, 1449 bp, Pseudomonas sp.
  misc_feature 1..1449: note = ribosomal RNA nucleic acid sequence
  source 1..1449: mol_type = genomic DNA
aatcatggctcagattgaacgctggcggcaggcctaacacatgcaagtcgagcggtagagaggtgcttgcacctcttgagagcggcggacgggtgagtaatgcctaggaatctgcctggtagtgggggataacgctcggaaacggacgctaataccgcatacgtcctacgggagaaagcaggggaccttcgggccttgcgctatcagatgagcctaggtcggattagctagttggtggggtaatggctcaccaaggcgacgatccgtaactggtctgagaggatgatcagtcacactggaactgagacacggtccagactcctacgggaggcagcagtggggaatattggacaatgggcgaaagcctgatccagccatgccgcgtgtgtgaagaaggtcttcggattgtaaagcactttaagttgggaggaagggcattaacctaatacgttagtgttttgacgttaccgacagaataagcaccggctaactctgtgccagcagccgcggtaatacagagggtgcaagcgttaatcggaattactgggcgtaaagcgcgcgtaggtggttcgttaagttggatgtgaaagccccgggctcaacctgggaactgcattcaaaactgtcgagctagagtatggtagagggtggtggaatttcctgtgtagcggtgaaatgcgtagatataggaaggaacaccagtggcgaaggcgaccacctggactgatactgacactgaggtgcgaaagcgtggggagcaaacaggattagataccctggtagtccacgccgtaaacgatgtcaactagccgttgggagccttgagctcttagtggcgcagctaacgcattaagttgaccgcctggggagtacggccgcaaggttaaaactcaaatgaattgacgggggcccgcacaagcggtggagcatgtggtttaattcgaagcaacgcgaagaaccttaccaggccttgacatccaatgaactttccagagatggattggtgccttcgggagcattgagacaggtgctgcatggctgtcgtcagctcgtgtcgtgagatgttgggttaagtcccgtaacgagcgcaacccttgtccttagttaccagcacgttatggtgggcactctaaggagactgccggtgacaaaccggaggaaggtggggatgacgtcaagtcatcatggcccttacggcctgggctacacacgtgctacaatggtcggtacagagggttgccaagccgcgaggtggagctaatcccacaaaaccgatcgtagtccggatcgcagtctgcaactcgactgcgtgaagtcggaatcgctagtaatcgcgaatcagaatgtcgcggtgaatacgttcccgggccttgtacacaccgcccgtcacaccatgggagtgggttgcaccagaagtagctagtctaaccttcgggaggacggttacca

SEQ ID NO: 14 - DNA, 1441 bp, Pseudomonas sp.
  misc_feature 73: note = n is a, c, g, or t
  misc_feature 107: note = n is a, c, g, or t
  misc_feature 235: note = n is a, c, g, or t
  misc_feature 1113: note = n is a, c, g, or t
  misc_feature 1115: note = n is a, c, g, or t
  misc_feature 1..1441: note = ribosomal RNA nucleic acid sequence
  source 1..1441: mol_type = genomic DNA
tcatggctcagattgaacgctggcggcaggcctaacacatgcaagtcgagcggatgagaggagcttgctcctngattcagcggcggacgggtgagtaatgcctaggnatctgcccagtagtgggggacaacgtttcgaaaggaacgctaataccgcatacgtcctacgggagaaagtgggggatcttcggacctcacgctattggatgagcctaggtcggattagctagttggtngggtaaaggcctaccaaggcgacgatccgtaactggtctgagaggatgatcagtcacactggaactgagacacggtccagactcctacgggaggcagcagtggggaatattggacaatgggcgaaagcctgatccagccatgccgcgtgtgtgaagaaggccctcgggtcgtaaagcactttaagttgggaggaagggcttacagcgaatacctgtgagttttgacgttaccaacagaataagcaccggctaacttcgtgccagcagccgcggtaatacgaagggtgcaagcgttaatcggaattactgggcgtaaagcgcgcgtaggtggcttgataagttggatgtgaaatccccgggctcaacctgggaactgcatccaaaactgtctggctagagtgcggtagagggtagtggaatttccagtgtagcggtgaaatgcgtagatattggaaggaacaccagtggcgaaggcgactacctggactgacactgacactgaggtgcgaaagcgtggggagcaaacaggattagataccctggtagtccacgccgtaaacgatgtcaactagccgttgggatccttgagatcttagtggcgcagctaacgcattaagttgaccgcctggggagtacggccgcaaggttaaaactcaaatgaattgacgggggcccgcacaagcggtggagcatgtggtttaattcgaagcaacgcgaagaaccttacctggccttgacatgctgagaactttccagagatggattggtgccttcgggaactcagacacaggtgctgcatggctgtcgtcagctcgtgtcgtgagatgttgggttaagtcccgtaacgagcgcaacccttgtccttagttaccagcacntnatggtgggcactctaaggagactgccggtgacaaaccggaggaaggtggggatgacgtcaagtcatcatggcccttacggccagggctacacacgtgctacaatggtcggtacaaagggttgccaagccgcgaggtggagctaatcccataaaaccgatcgtagtccggatcgcagtctgcaactcgactgcgtgaagtcggaatcgctagtaatcgtgaatcagaacgtcacggtgaatacgttcccgggccttgtacacaccgcccgtcacaccatgggagtgggttgctccagaagtagctagtctaaccttcgggaggacgg

SEQ ID NO: 15 - DNA, 1376 bp, Gluconobacter sp.
  misc_feature 1..1376: note = ribosomal RNA nucleic acid sequence
  source 1..1376: mol_type = genomic DNA
cggcatgcttaacacatgcaagtcgcacggatctttcgggattagtggcggacgggtgagtaacgcgtagggatctatccatgggtgggggacaactccgggaaactggagctaataccgcatgatacctgagggtcaaaggcgcaagtcgcctgtggaggaacctgcgttcgattagctagttggtggggtaaaggcctaccaaggcgatgatcgatagctggtttgagaggatgatcagccacactgggactgagacacggcccagactcctacgggaggcagcagtggggaatattggacaatgggcgaaagcctgatccagcaatgccgcgtgtgtgaagaaggtcttcggattgtaaagcactttcgacggggacgatgatgacggtacccgtagaagaagccccggctaacttcgtgccagcagccgcggtaatacgaagggggctagcgttgctcggaatgactgggcgtaaagggcgcgtaggcggttgatgcagtcagatgtgaaatccccgggcttaacctgggaactgcatttgagacgcattgactagagttcgagagagggttgtggaattcccagtgtagaggtgaaattcgtagatattgggaagaacaccggtggcgaaggcggcaacctggctcgatactgacgctgaggcgcgaaagcgtggggagcaaacaggattagataccctggtagtccacgctgtaaacgatgtgtgctggatgttgggtaacttagttactcagtgtcgaagctaacgcgctaagcacaccgcctggggagtacggccgcaaggttgaaactcaaaggaattgacgggggcccgcacaagcggtggagcatgtggtttaattcgaagcaacgcgcagaaccttaccagggcttgcatggggaggacgtactcagagatgggtatttcttcggacctcccgcacaggtgctgcatggctgtcgtcagctcgtgtcgtgagatgttgggttaagtcccgcaacgagcgcaacccttgtctttagttgccagcactttcaggtgggcactctagagagactgccggtgacaagccggaggaaggtggggatgacgtcaagtcctcatggcccttatgtcctgggctacacacgtgctacaatggcggtgacagtgggaagctatgtggtgacacagtgctgatctctaaaagccgtctcagttcggattgtactctgcaactcgagtacatgaaggtggaatcgctagtaatcgcggatcagcatgccgcggtgaatacgttcccgggccttgtacacaccgcccgtcacaccatgggagttggttcgaccttaagccggtgagcgaaccgcaaggacgcagccgaccacggac

SEQ ID NO: 16 - DNA, 1289 bp, Bacillus sp.
  misc_feature 39: note = n is a, c, g, or t
  misc_feature 64: note = n is a, c, g, or t
  misc_feature 1076: note = n is a, c, g, or t
  misc_feature 1092: note = n is a, c, g, or t
  misc_feature 1..1289: note = ribosomal RNA nucleic acid sequence
  source 1..1289: mol_type = genomic DNA
tgcaagtcgagcggagttttgaaaagcttgcttttcaanacttagcggcggacgggtgagtaanacgtgggcaacctgcccttgagacggggataactccgggaaaccggagctaataccggataacacatatcttcgcatgaggatatgttagaaggtggcttttagctaccactcaaggatgggcccgcggcgcattagctagttggtgaggtaacggctcaccaaggcgacgatgcgtagccgacctgagagggtgatcggccacactgggactgagacacggcccagactcctacgggaggcagcagtagggaatcttccgcaatggacgaaagtctgacggagcaacgccgcgtgagtgatgaaggttttcggatcgtaaagctctgttgttagggaagaacaagtacctgttaaataagcaggtaccttgacggtacctaaccagaaagccacggctaactacgtgccagcagccgcggtaatacgtaggtggcaagcgttgtccggaattattgggcgtaaagcgcgcgcaggcggttccttaagtctgatgtgaaagcccacggctcaaccgtggagggtcattggaaactggggaacttgagtgcagaagaggagagcggaattccacgtgtagcggtgaaatgcgtagagatgtggaggaacaccagtggcgaaggcggctctctggtctgtaactgacgctgaggcgcgaaagcgtggggagcgaacaggattagataccctggtagtccacgccgtaaacgatgagtgctaagtgttagagggtttccgccctttagtgctgcagcaaacgcattaagcactccgcctggggagtacggtcgcaagactgaaactcaaaggaattgacggggacccgcacaagcggtggagcatgtggtttaattcgaagcaacgcgaagaaccttaccaggtcttgacatcctctgctacttctagagatagaaggttcccttcggggacagagtgacaggtggtgcatggttgtcgtcagctcgtgtcgtgagatgttgggttaagtcccgcaacgagcgcaacccttgatnttagttgccagcattnagttgggcactctaaggtgactgccggtgacaaaccggaggaaggtggggatgacgtcaaatcatcatgccccttatgacctgggctacacacgtgctacaatggatggtacaaagggctgcaaaaccgcgaggttaagccaatcccataaaaccattctcagttcggattgtaggctgcaactcgcctacatgaag

SEQ ID NO: 17 - DNA, 1414 bp, Enterobacter sp.
  misc_feature 973: note = n is a, c, g, or t
  misc_feature 1141: note = n is a, c, g, or t
  misc_feature 1164: note = n is a, c, g, or t
  misc_feature 1207: note = n is a, c, g, or t
  misc_feature 1245: note = n is a, c, g, or t
  misc_feature 1258: note = n is a, c, g, or t
  misc_feature 1272: note = n is a, c, g, or t
  misc_feature 1284: note = n is a, c, g, or t
  misc_feature 1353: note = n is a, c, g, or t
  misc_feature 1357: note = n is a, c, g, or t
  misc_feature 1..1414: note = ribosomal RNA nucleic acid sequence
  source 1..1414: mol_type = genomic DNA
agagtttgatcatggctcagattgaacgctggcggcaggcctaacacatgcaagtcgaacggtagcacagagagcttgctctcgggtgacgagtggcggacgggtgagtaatgtctgggaaactgcctgatggagggggataactactggaaacggtagctaataccgcataacgtcgcaagaccaaagagggggaccttcgggcctcttgccatcagatgtgcccagatgggattagctagtaggtggggtaacggctcacctaggcgacgatccctagctggtctgagaggatgaccagccacactggaactgagacacggtccagactcctacgggaggcagcagtggggaatattgcacaatgggcgcaagcctgatgcagccatgccgcgtgtatgaagaaggccttcgggttgtaaagtactttcagcggggaggaaggtgttgtggttaataaccgcagcaattgacgttacccgcagaagaagcaccggctaactccgtgccagcagccgcggtaatacggagggtgcaagcgttaatcggaattactgggcgtaaagcgcacgcaggcggtctgtcaagtcggatgtgaaatccccgggctcaacctgggaactgcattcgaaactggcaggctagagtcttgtagaggggggtagaattccaggtgtagcggtgaaatgcgtagagatctggaggaataccggtggcgaaggcggccccctggacaaagactgacgctcaggtgcgaaagcgtggggagcaaacaggattagataccctggtagtccacgccgtaaacgatgtcgacttggaggttgtgcccttgaggcgtggcttccggagctaacgcgttaagtcgaccgcctggggagtacggccgcaaggttaaaactcaaatgaattgacgggggcccgcacaagcggtggagcatgtggtttaattcgatgcaacgcgaagaacctnacctactcttgacatccagagaacttagcagagatgctttggtgccttcgggaactctgagacaggtgctgcatggctgtcgtcagctcgtgttgtgaaatgttgggttaagtcccgcaacgagcgcaacccttatcctttgttgccagcggtccggccgggaactcnaaggagactgccagtgataaacnggaggaaggtggggatgacgtcaagtcatcatggcccttacgngtagggctacacacgtgctacaatggcgcatacaaagngaagcgaactcgngagagcaagcgganctcataaagtgngtcgtagtccggattggagtctgcaactcgactccatgaagtcggaatcgctagtaatcgtagatcagnatgntacggtgaatacgttcccgggccttgtacacaccgcccgtcacaccatgggagtggg

SEQ ID NO: 18 - DNA, 1522 bp, Enterobacter sp.
  misc_feature 1..1522: note = ribosomal RNA nucleic acid sequence
  source 1..1522: mol_type = genomic DNA
agagtttgatcatggctcagattgaacgctggcggcaggcctaacacatgcaagtcgaacggtagcacagagagcttgctctcgggtgacgagtggcggacgggtgagtaatgtctgggaaactgcctgatggagggggataactactggaaacggtagctaataccgcataacgtcgcaagaccaaagagggggaccttcgggcctcttgccatcagatgtgcccagatgggattagctagtaggtggggtaacggctcacctaggcgacgatccctagctggtctgagaggatgaccagccacactggaactgagacacggtccagactcctacgggaggcagcagtggggaatattgcacaatgggcgcaagcctgatgcagccatgccgcgtgtatgaagaaggccttcgggttgtaaagtactttcagcggggaggaaggtgttgtggttaataaccgcagcaattgacgttacccgcagaagaagcaccggctaactccgtgccagcagccgcggtaatacggagggtgcaagcgttaatcggaattactgggcgtaaagcgcacgcaggcggtctgtcaagtcggatgtgaaatccccgggctcaacctgggaactgcattcgaaactggcaggctagagtcttgtagaggggggtagaattccaggtgtagcggtgaaatgcgtagagatctggaggaataccggtggcgaaggcggccccctggacaaagactgacgctcaggtgcgaaagcgtggggagcaaacaggattagataccctggtagtccacgccgtaaacgatgtcgacttggaggttgtgcccttgaggcgtggcttccggagctaacgcgttaagtcgaccgcctggggagtacggccgcaaggttaaaactcaaatgaattgacgggggcccgcacaagcggtggagcatgtggtttaattcgatgcaacgcgaagaaccttacctactcttgacatccagagaacttagcagagatgctttggtgccttcgggaactctgagacaggtgctgcatggctgtcgtcagctcgtgttgtgaaatgttgggttaagtcccgcaacgagcgcaacccttatcctttgttgccagcggtccggccgggaactcaaaggagactgccagtgataaactggaggaaggtggggatgacgtcaagtcatcatggcccttacgagtagggctacacacgtgctacaatggcgcatacaaagagaagcgaactcgcgagagcaagcggacctcataaagtgcgtcgtagtccggattggagtctgcaactcgactccatgaagtcggaatcgctagtaatcgtagatcagaatgctacggtgaatacgttcccgggccttgtacacaccgcccgtcacaccatgggagtgggttgcaaaagaagtaggtagcttaaccttcgggagggcgcttaccactttgtgattcatgactggggtgaagtcgtaacaaggtaaccgtaggggaacctgcggttgga

SEQ ID NO: 19 - DNA, 1433 bp, Pseudomonas sp.
  misc_feature 1115: note = n is a, c, g, or t
  misc_feature 1..1433: note = ribosomal RNA nucleic acid sequence
  source 1..1433: mol_type = genomic DNA
tcatggctcagattgaacgctggcggcaggcctaacacatgcaagtcgagcggtagagagaagcttgcttctcttgagagcggcggacgggtgagtaatgcctaggaatctgcctggtagtgggggataacgttcggaaacggacgctaataccgcatacgtcctacgggagaaagcaggggaccttcgggccttgcgctatcagatgagcctaggtcggattagctagttggtgaggtaatggctcaccaaggcgacgatccgtaactggtctgagaggatgatcagtcacactggaactgagacacggtccagactcctacgggaggcagcagtggggaatattggacaatgggcgaaagcctgatccagccatgccgcgtgtgtgaagaaggtcttcggattgtaaagcactttaagttgggaggaagggttgtagattaatactctgcaattttgacgttaccgacagaataagcaccggctaactctgtgccagcagccgcggtaatacagagggtgcaagcgttaatcggaattactgggcgtaaagcgcgcgtaggtggtttgttaagttggatgtgaaatccccgggctcaacctgggaactgcattcaaaactgactgactagagtatggtagagggtggtggaatttcctgtgtagcggtgaaatgcgtagatataggaaggaacaccagtggcgaaggcgaccacctggactaatactgacactgaggtgcgaaagcgtggggagcaaacaggattagataccctggtagtccacgccgtaaacgatgtcaactagccgttggaagccttgagcttttagtggcgcagctaacgcattaagttgaccgcctggggagtacggccgcaaggttaaaactcaaatgaattgacgggggcccgcacaagcggtggagcatgtggtttaattcgaagcaacgcgaagaaccttaccaggccttgacatccaatgaactttctagagatagattggtgccttcgggaacattgagacaggtgctgcatggctgtcgtcagctcgtgtcgtgagatgttgggttaagtcccgtaacgagcgcaacccttgtccttagttaccagcacgtnatggtgggcactctaaggagactgccggtgacaaaccggaggaaggtggggatgacgtcaagtcatcatggcccttacggcctgggctacacacgtgctacaatggtcggtacagagggttgccaagccgcgaggtggagctaatcccataaaaccgatcgtagtccggatcgcagtctgcaactcgactgcgtgaagtcggaatcgctagtaatcgcgaatcagaatgtcgcggtgaatacgttcccgggccttgtacacaccgcccgtcacaccatgggagtgggttgcaccagaagtagctagtctaaccttcgg

SEQ ID NO: 20 - DNA, 1487 bp, Bacillus sp.
  misc_feature 160: note = n is a, c, g, or t
  misc_feature 265: note = n is a, c, g, or t
  misc_feature 1231: note = n is a, c, g, or t
  misc_feature 1..1487: note = ribosomal RNA nucleic acid sequence
  source 1..1487: mol_type = genomic DNA
tggctcaggacgaacgctggcggcgtgcctaatacatgcaagtcgagcggacagatgggagcttgctccctgatgttagcggcggacgggtgagtaacacgtgggtaacctgcctgtaagactgggataactccgggaaaccggggctaataccggatgnttgtttgaaccgcatggttcagacataaaaggtggcttcggctaccacttacagatggacccgcggcgcattagctagttggtgaggtaacggctcaccaaggcnacgatgcgtagccgacctgagagggtgatcggccacactgggactgagacacggcccagactcctacgggaggcagcagtagggaatcttccgcaatggacgaaagtctgacggagcaacgccgcgtgagtgatgaaggttttcggatcgtaaagctctgttgttagggaagaacaagtgccgttcaaatagggcggcaccttgacggtacctaaccagaaagccacggctaactacgtgccagcagccgcggtaatacgtaggtggcaagcgttgtccggaattattgggcgtaaagggctcgcaggcggtttcttaagtctgatgtgaaagcccccggctcaaccggggagggtcattggaaactggggaacttgagtgcagaagaggagagtggaattccacgtgtagcggtgaaatgcgtagagatgtggaggaacaccagtggcgaaggcgactctctggtctgtaactgacgctgaggagcgaaagcgtggggagcgaacaggattagataccctggtagtccacgccgtaaacgatgagtgctaagtgttagggggtttccgccccttagtgctgcagctaacgcattaagcactccgcctggggagtacggtcgcaagactgaaactcaaaggaattgacgggggcccgcacaagcggtggagcatgtggtttaattcgaagcaacgcgaagaaccttaccaggtcttgacatcctctgacaatcctagagataggacgtccccttcgggggcagagtgacaggtggtgcatggttgtcgtcagctcgtgtcgtgagatgttgggttaagtcccgcaacgagcgcaacccttgatcttagttgccagcattcagttgggcactctaaggtgactgccggtgacaaaccggaggaaggtggggatgacgtcaaatcatcatgccccttatgacctgggctacacacgtgctacaatggncagaacaaagggcagcgaaaccgcgaggttaagccaatcccacaaatctgttctcagttcggatcgcagtctgcaactcgactgcgtgaagctggaatcgctagtaatcgcggatcagcatgccgcggtgaatacgttcccgggccttgtacacaccgcccgtcacaccacgagagtttgtaacacccgaagtcggtgaggtaaccttttaggagccagccgccgaaggtgggacagatgattggggtgaagtcgt

SEQ ID NO: 21 - DNA, 491 bp, Serratia sp.
  misc_feature 1..491: note = Marker nucleic acid sequence
  source 1..491: mol_type = genomic DNA
gtgcgaccaggtcgtggcgtgcactgaggtagatcgccacgcccagcgcagcgagcaccacggtggctaccgtggcgaacagcacgatcagccgggtggcgatggaaaggcgcggtctcatgcgttgcgcgccgtggcgtcctcgggtgcctccagcacgtagcccatgccgcgcaccgtcacgatcagcttgtcgatgaagtcgtcgtcgatcttcgcgcgcaggcggcggatcgccacgtcgatgacgttggtatcactgtcgaaattcatgtcccagacctgcgaggcgatcaacgaacgtggcagcacttcgccacggcgacgtgcaagcagctccagcagggtgtattccttcgggctgagcgtgatgcgctggccgttgcgttccacccgccggcgcagggtgtcgaccaccaggtcggcgaccacgatccgttcggccagcggcgttgcctggccacgccgcagcagggtgcgcacacgggcca

SEQ ID NO: 22 - DNA, 451 bp, Serratia sp.
  misc_feature 1..451: note = Marker nucleic acid sequence
  source 1..451: mol_type = genomic DNA
agcgccgcgcgagggcctgcgcactctcatatccagcggccagcgcagcgtcggtgacgcttgcatcgggctgctgcagcgcctgcagggcgttgagcaggcgcagccggtccagcgtctgtccggggctttccccggtaagtgcccggtacaggcgctggaagtgatagggcgactgatgggcgacagtggccagtgacgccacatccggcagtgcctgctgctcacgcaggcagccctgcagatggtcgatgacccgttcgattccctgcgcctggcgcaggcctgcaagccgcttcatgaccatctccgctgaggacctggctgcgatcgtgcctgatcctttagcggggtgcgtgaccgatcctgcgcgattgcccgccctcaggcctgggcgagagcctgttccaggtccgcgcgcagatcgccgatgtgctcgatgccgatcgac

SEQ ID NO: 23 - DNA, 449 bp, Serratia sp.
  misc_feature 1..449: note = Marker nucleic acid sequence
  source 1..449: mol_type = genomic DNA
cggaatggcgacgcgcctggcctcgcacctgccggggtacatgatccccagtcactacgtgcttgtggaccggttcccgtacctgcccaatggcaaggtcgatcgggctacgcttctggcgatggcgccggcacaccttgcccagagccaggcgataccaccgcgcgacgccaccgagcgcgggctgctgacgatatggggcgagctgctgggccgcgacgatctgggcatcgagcacgacttcttcagggcgggtgggcactccctgctggcgacccagctggtcgctcgggtgcgcgacaccttcgcggtggacatcagtgtccgcgatctgttcacccatgccaccattgcgagcctggccgcgcggatcgccgaggcgctcccggtcgctgccgacgcgcgcccggccccgctcgcgtcatccgtgctgcgggcatcgggcaccg

SEQ ID NO: 24 - DNA, 446 bp, Serratia sp.
  misc_feature 1..446: note = Marker nucleic acid sequence
  source 1..446: mol_type = genomic DNA
aaggtgatggacatggccgaacaggtggccggcaccgacatcaacattctgctgaccggcgagaacgggacaggcaagagcatgctagcttcgttgatccacgagcgttcaaggcgcgcgcagagcgcgttcgtggccatcaacatgagcgcgattccggacacgctgttcgaaagtgaactgtacggccatgtcaagggcgcgttcaccgatgcgcgcagcaaccgcatggggcgctttgaactggccgagggcggcacgctgttcatggatgaaatcggtgacctgccggcggtgcagcaggccaaactcctgcatgtactggaatcgcggcagtacgagaagctgggctgcagccatagccgcgttgccgacgtccgcatcatcgcagcaaccaatgccgaccttccggcgctggtcgacaatggccggttccgccgcgatct

SEQ ID NO: 25 - DNA, 436 bp, Serratia sp.
  misc_feature 1..436: note = Marker nucleic acid sequence
  source 1..436: mol_type = genomic DNA
cgacgacgcgttcgaaaggcaggtcctgatgtgcgtatgcgtcggtcaacgtagcgcgcactgcatccagatatgccaggaaaggcatgtccggttccatcctgctgcgtaccgccagggtgttgacgaagtagccgatcaggggctcaagctcgcgctggggtcgattcagcgtcgacacgcccaccacgaaatcctcctgctgcgacgtgcgccacagcggcagttgccagctggccagaagcagcatgaacggggttgtgcccgcgtttcgggccagcgcattcacgcgggcactaagtgcggcgtccagttcgaagggcacggaccctccgcgcaggtccaactgggcgggccgcgggtagtccgtcggaagctccagggtgtgcggtacgccgtcaagctgccgcatccagtacgccaactggcgctcgag

SEQ ID NO: 26 - DNA, 320 bp, Pseudomonas sp.
  misc_feature 1..320: note = Marker nucleic acid sequence
  source 1..320: mol_type = genomic DNA
gcccgctcagtggcgggctgctattcggtttcgagggtggtcggtggcggcggcgtttccggttgcggcatctccagccgcacgtcgatccagctgttgagcggcacgtccagcggagccccgcggccggggatcatttcgccgtcttcggacagggtccagcgttgcttgaacaggcgaattgtcacagtgccgtcggcgtcctgctcgctctcagtgatgccgagcgtgccaccgccatctggtgagcacgggtcttgaatgcgccagccttccagggcaaggcccaggctgccggtcacgcggtactcaccgacgcc

SEQ ID NO: 27 - DNA, 320 bp, Pseudomonas sp.
  misc_feature 1..320: note = Marker nucleic acid sequence
  source 1..320: mol_type = genomic DNA
gcccgctcagtggcgggctgctattcggtttcgagggtggtcggtggcggcggcgtttccggttgcggcatctccaggcgcacgtcgatccagctgttgagtggcacgtccagcggagccccgcggccggggatcatttcgccgtcttcggacagggtccagcgttgcttgaacagccggatgacaacagtgccgtcatcgtcttgctcgctctcggtgatgccgagcgtgccaccaccgtccggtgagcacgggtcttgaatgcgccagccttccagggcaaggcccaggctgccggtcacgcggtactcaccgacgcc

SEQ ID NO: 28 - DNA, 374 bp, Streptomyces sp.
  misc_feature 1..374: note = Marker nucleic acid sequence
  source 1..374: mol_type = genomic DNA
ctggaccttggctacgccaagaccaccacgctggccttcacggccgcgggcaacaactttgaactggccatcgccgtggcgattggcaccttcggtgtgacgtccggccaagcccttgccggcgtcgtcggccccttgattgaagtgccggcacttgttgcacttgtatacgccgcactgtgggcgcgaaagcgcttcttcagctccgccaccgcttcactctgaccaccgccataaccctggagaacaccatgaccaccgaatctgccaagaagccctccgtcctgttcgtctgcgtccacaacgccggccgctcacagatggccgccgccttcctcaccagcctctccaagggtgcgatcgaggtgcgctcc

SEQ ID NO: 29 - DNA, 365 bp, Streptomyces sp.
  misc_feature 1..365: note = Marker nucleic acid sequence
  source 1..365: mol_type = genomic DNA
gccagacggaccaaggccctggtgtcgccgtggtcggcggcgcgttgggcgagggtttcggcgccctgccggtcaccctccagctcccgcatcccggccagatcgaccaaggccctggtgccgccgtggtcggcggcgcgttgggcgagggcttcggcgccctctcggtcccccgccctctcccgcatcccggccagatcgaccaaggccccggtgccgccatggtcggcggcacgctgcaagagaacttcggcgccctgccggtcgccctccaacttccgcatcccagccagacggaccaaggccctggtgtcgccgtggtcggcggcgcgttgggcgagggtttcggcgccctgccggtcacc

SEQ ID NO: 30 - DNA, 344 bp, Streptomyces sp.
  misc_feature 1..344: note = Marker nucleic acid sequence
  source 1..344: mol_type = genomic DNA
ccgtgaacttccaccgcgcggtgttctccggcggcaccgtggacttcggccgcgcggcgttctccggcggcaccgtgcacttcggccgcgcggcgttctccggcagcaccgtgcacttcagcggcgcggcgttctccggcagcaccgtgcacttcagcggcgcggcgttctccggcggcgccgtgaacttcggcggcgcgaggttctccggcggcaccgtgaacttcggcggcgcggcgttctccggcggcaccgtgcacttcggcctcgcggcgttctccggcggcaccgtggacttcggccgcgcggcgttctccgacggcaccgtgcacttccgcgacgcg

SEQ ID NO: 31 - DNA, 308 bp, Streptomyces sp.
  misc_feature 1..308: note = Marker nucleic acid sequence
  source 1..308: mol_type = genomic DNA
tgctcccccgcggtgcggggggcgggccggagtcgcggtgccggtcggcctcgtgggccccggctccgcgagcgggccgtcagtgcgtgaggatcttcgagaggaagtcgcgggcgcgctcggacttcggcgcggtgaagaactcctccggcgtggcctcctcgacgatctggccctcggccatgaacacgacgcggtcggcggccttgcgggcgaagcccatctcgtgggtgacgacgatcatcgtcatgccgtcggccgcgagctgcaccatgacgtcgagcacctcggtgatcatctcggggtcg

SEQ ID NO: 32 - DNA, 289 bp, Streptomyces sp.
  misc_feature 1..289: note = Marker nucleic acid sequence
  source 1..289: mol_type = genomic DNA
cctcgtacgaccggacgaacgcgagcaccgactcctggtccgtctcggccacctcgagggtgccgagcccgaagaccgggtgggccttgcggacgtggatgacgttccgcacccagtgcagcagcgagcgcgactgtgcgagctggctctcgacgttgacgaggttgtagttgaagacgagcgactgcacgacgggcaggaacagcttgcccgggtcggcggtcgagaagccggcgttgcggtcgggcgtccactgcatcggggtgcgggacgagtcgcggtcgggcag

SEQ ID NO: 33 - DNA, 428 bp, Pseudomonas sp.
  misc_feature 1..428: note = Marker nucleic acid sequence
  source 1..428: mol_type = genomic DNA
gcatcgaggtggacgaaggcgctgggcaccatgtattcaggcaggtgcttgagcagggcgctgcgcaggtgttcggcgttggccggttcaccgcacaggtacgccaccaggcgattatcctcgcgagcgatcaccacggcatcggtgacaccggcacagccgagcaagacgttctcgatctcgcccaactcgatacggaagccacgaatcttcacctggaagtcattgcgcccgaggtactccaatgtgccgtcggccagccaacgacccaggtcgccggtcttgtacagccgtgcgttcggcgcggtgctgaacgggtcggcaacaaagcgctcggcgctcagttccggccggttcaggtaaccccgggccacgccagcgccgccaatgtgcagttcaccagccacgcccaacggcgtcggttcacc

SEQ ID NO: 34 - DNA, 381 bp, Pseudomonas sp.
  misc_feature 1..381: note = Marker nucleic acid sequence
  source 1..381: mol_type = genomic DNA
acgaagaatggcaggtattgctgggcagcggctcggcgcaaatcgatgtcgtcagcggtttgctgacatttaaccctaccgggccggacaagtttttggtcattactgtcctggtacccccttcgaggccaagtgcggcttcggaggatggttacatcgtcctgccgttgccgttattcagtgtgcccgaaacgatccagatgttccgtgctgatggtcagtaagtggcccggaccctaaaccgtgagcatccggattcagatggtgagttcatgctcaaccaaaggattacttccatggaaatcaactctgtagatgcgctgctggactggcttaaagtaaaacctcggactctggactggggggcgattctggcctatg

SEQ ID NO: 35 - DNA, 354 bp, Pseudomonas sp.
  misc_feature 1..354: note = Marker nucleic acid sequence
  source 1..354: mol_type = genomic DNA
ggttctaacttgcagacgtctgcagcgaagttaacgatgaaagaggtcggcggtacccacctgtctttcactaaacaagaaggtgcccaacaatggtcgctcactcggatttccgagaaaaacgtactggatggtccggggttgaagtttaatatcaatcttatggcgagcacggggtcggttacctcggcggggcgagtggaactcaatatctcggagggtagtaactatcggttgattgacatgccgtccgagcacttgcaaagggttgctggtcaacgtttccagacgcacttcagggcgttaccggaggaccagaaagtttttgtactgaacgaattgaagtttgagccg

SEQ ID NO: 36 - DNA, 341 bp, Pseudomonas sp.
  misc_feature 1..341: note = Marker nucleic acid sequence
  source 1..341: mol_type = genomic DNA
ttccaccaatacgccgccggactgatgccggtgttcgcccaattgcgctacctgatcgtcggcggcgatgtgctcgatccgaccgtgatcggccgtgtcctgaaagagggcgcaccgctgcacctgctcaacggctacggcccgaccgaggccaccactttcaccaccacctacgaaatcaagcaggtcggcgagggcggtatcccgatcggtcgtccgattggcaacacccgcgtctatgtgctggacgccaatcaacaaccagtgcccatcggtgtggccggcgagttgtacatcggtggcgacggcgtggcgaaagggtatctgaatcgccctgagct

SEQ ID NO: 37 - DNA, 207 bp, Pseudomonas sp.
  misc_feature 1..207: note = Marker nucleic acid sequence
  source 1..207: mol_type = genomic DNA
gcgatcaccagcagatcgctttccagttgttcagccagcagcgccgagcacaggtctttgtcgatcacggcttccacgccttgtagcttgccgtcggcgtcgtacatcgtcgggatgccgccaccgccggcaagcccttgcttccacagttctgctccggagagcgcgaactgcatgaggtcctagatatccgccaacgccgccacc

SEQ ID NO: 38 - DNA, 569 bp, Pseudomonas sp.
  misc_feature 1..569: note = Marker nucleic acid sequence
  source 1..569: mol_type = genomic DNA
ctgggcaacaccctgaccatcaccggcttcaacgctgctaccggtgtagtgagctacagctacacgcttctcgacaatgaagcccatccaaacgccaacggtgccaacagcgttagcgagcaatttgccgtagtcgccaccgatgacaacggcaccaccgccaacggcaacctcgatgtgaacatcgtcgatgacctgcccaacgccgtggacgacagcaacggtaccgcctcggaaaccaacctgaccctgaccggcagcgtgctgaccaacgacacccaaggtgcggaccctgtggcgtccggcccaatcacccccggcaccttcaccggcacttacggcaccttggtgctcaacgccgacggttcctacacctacaccctgaacaccgccgacgccgacttcaaaggcttgcacggcggcggcaatggcagcgaaaccttcacttacaccctgaccgatgcggatggcgacaccagcaccgcgaacctggtcttgcaggtgcacaacaacgacgacccggtgatcatcaccggcctcgacaccgaaggcggcgagctgtcgttgca

SEQ ID NO: 39 - DNA, 474 bp, Pseudomonas sp.
  misc_feature 1..474: note = Marker nucleic acid sequence
  source 1..474: mol_type = genomic DNA
acataaaccggccgaacccccgaatccgccggaaacactagaatgaaatccctgtactccggcggatagatcggatcgacaatgatgctgtcggccatcggcgtcggcgggtagatccaaataggcggtgcctggggcgcagcttccagggcgggaatgccgagggtgtcagccggattgatagccggcgtccagatcagttcgatgccatcacccaggtcagcaatgaactgatcggctcgcgacgtgaactgaacaacatcaaccatttcccaatcgggatgctggccggtgtagaagccataccccttgaggctgccgtcggcctgctgctcgacgctcaagcgcatgcgactgcgggcttgtttgaggtcgcgtagctggtcttcgctataaagcgcgctgtcacctagattggacggccagagcagggcgacgatgccggtcagcaacgctgcgccgacggtgccgccc

SEQ ID NO: 40 - DNA, 407 bp, Pseudomonas sp.
  misc_feature 1..407: note = Marker nucleic acid sequence
  source 1..407: mol_type = genomic DNA
tacaggttgtacaggccaacatgcggcagttgcgtcttgaaacgccgcaccagatgccccggcaaggcctcgccgctgcacatcacccgcaccaagccttcgcactgacccgcttcgccatgggccaggaacacatcgagcatcgacggcacaaagtgcagcgtggtgatgccttgggcctggatcacttcgcgcaggtacgccgggtcgcgatgcccgccaggacgggccattaccagccgcgcgccgctgaacagcggccagaagaactcccacaccgacacgtcgaagctgaacggggtcttttgcagcaccgcgtctgtggcgctcaagccgtattcgtcctgcatccacagcaaacggttgaccaccgcgccgtgctcgttcatcacgcccttgggcaggcc

SEQ ID NO: 41 - DNA, 392 bp, Pseudomonas sp.
  misc_feature 1..392: note = Marker nucleic acid sequence
  source 1..392: mol_type = genomic DNA
taggtccacaccgccttgccacgctgacgggtgtgcaggaaaccgttacggtattcgtaggacgtcggcgcctcgtccggaggaatcaacgccagcagccgtccgacctcgtcgtagcggtattcgcggaccgcccccagcgggtcctgttcggcgatcaaccggccctgttcgtcataggccttgaggtgctcgccgccgtcgggctcgaccttgcgcaccagccgcgcccggtcgtcgtggacgtacacttcctggctaccatccaggtgccgaaccgtgacgctgccgtcctcaccccaggtgtagcggctgtccatctgcgcgaacgaggcccagtgccggacacagcgggacgccggcccgacgtcttgccactcccaataaaaact

SEQ ID NO: 42 - DNA, 379 bp, Pseudomonas sp.
  misc_feature 1..379: note = Marker nucleic acid sequence
  source 1..379: mol_type = genomic DNA
caatacgcataagcattaatccccccatcaccaaaaggactcaactcatccgggctattgaaccgcatcaacaccggattaaaagcccgattaccctgtcccaataaataatgccccgttaccggatcggggcgctcgccattgaacccgagcaaactgctcaagccactttccgcaggccgatgaccataggcggtatacgccatcggctgggtatcagtgccagccagcgtctgcaaaaccgaccgctgctggtccgttgccaacagcgtcgtctcggtgacattggcgatgtgcaagcgttgcgccaggggctgggcttcatggcgaaggatggtgagttccacctggccttcgatttcattgaccagctcgtcgt

SEQ ID NO: 43 - DNA, 499 bp, Pantoea sp.
  misc_feature 1..499: note = Marker nucleic acid sequence
  source 1..499: mol_type = genomic DNA
cgccgacccgggagggctcgcgccggatcgcggaggtccgcggcccgaaggacctggagggcatcgacgtgaccgcgcgggggagcggcgtcggcaccggcggcatggtgaccaagctggagtccgtcgcgatcgccaccgcgtcgggcatcccggtcgtgctgacgtccaccgaccaggtcgccccggccctggacggcgccgacgtcggcacctggttcgccgccaccggcaagcgcgcctccacccggctgatgtggctcgcgtacgccgcgcggacccacggccggctggtgctggacgacggggccgtgcgggccgtcgtcgagcgcgggacgtcactgctgcccgccggggtcacggcggtcgagggcgagttcgaggccggcgacccggtcgagatcgtcggcgcggacggcacggtcgtcgcccgcgggctggtggcctactcgtcgcaggaggcgcccgagctgctcggccgcagcacgaacgagctgcg

SEQ ID NO: 44 - DNA, 487 bp, Pantoea sp.
  misc_feature 1..487: note = Marker nucleic acid sequence
  source 1..487: mol_type = genomic DNA
atcggcgcgggcggcaacgcgggcacgcagatcacggccacggtgatccgggcgatggccaccggcagcgtgcggctccgggacgcgggcgccgtcgtccgcaaggagctggtcaccgggctgatggtggcgggcacgatcgccgtggtcggctgggtgcgggcctggacgctcggcgtcggcggggaggtggcgctgacggtcgccgtgtccgcgggcgcgatcatcatctggtcggcgctggtggcgtccgtgctgccgctggtgctgcgcaaggtgggcctggaccccgcggtggggtcggggccgctgatcacgaccgtggtcgacggcaccgggctgatcatctacttcacggtggcacggctgctgatcacggcgctccagggctgaccggcgccgcgccgtagggtgtgcgcgtgcaggacgagacgagcagcgcaccggcgtcgccggtcgagagcgtcgaccgcgcgctgcgcacgct

SEQ ID NO: 45 - DNA, 484 bp, Pantoea sp.
  misc_feature 1..484: note = Marker nucleic acid sequence
  source 1..484: mol_type = genomic DNA
aactcgtcgagttcggcctggtagctgcagagctgggccgtgcagaccgccgtcgcgtcgcccgggtagaaggccagcaccacggtgcggccgatctcggcggacaggtcgtactcgtcgtcggtgcggacgccgccgcgcacgaccatccccggcagggtgaacgacggggcggactcgccgatcgcggggatgctcatgggtctcacggtagggcggcccggcggtggttgcccctcggcgcgctgtgcgggggctgtggatgcgctccgcggcctacgagaacaactgcgggaacgcgtgcgccacccaggggtacccgacgaagaccaccgcgtcgagcagcgcgtgcgtgatgacgagcggcaggagccggccccacctcgtgtagatccagccgaacacgatgcccatcaccgcgttgccgatgaacgccccgaacccctggtacaagtggtagctgccgcgcagcagggcggtcgac

SEQ ID NO: 46 - DNA, 480 bp, Pantoea sp.
  misc_feature 1..480: note = Marker nucleic acid sequence
  source 1..480: mol_type = genomic DNA
ggtcgtcgagcggggtccgtcggacgcggtcatcctcgacccgcaccacgactacacccggctgctcgccgaggccgcccccgacccggagcgcaccgagcgccggatcaccgcggggccgccgctcgaccggacgaagatcgacaacaccacctgctacgaccacacgatcggggactgggtgtcgagcgaggccgcaccggtcggggcgcgatgagcgacgggccgacgttcgtcgactgggtcaccgacgggttcgcggcacggttccgggtcggtgcggaccagccagcggcgctcgtgtcgttcgtgccggccggcggagcgtcggccggcagagcgctcgccgacgggccggacgacccgcagtcgctcgtggagctgacgacgatcgggcacgggcggttcccgggcgggttccggcacgtggactccaccatcggggcgcgactgcgccccgtgtcgcaccacgtgcacgac

SEQ ID NO: 47 - DNA, 480 bp, Pantoea sp.
  misc_feature 1..480: note = Marker nucleic acid sequence
  source 1..480: mol_type = genomic DNA
ggggccgaacgtcagcggggtggtcgcgtaggtcgcggtgccgtcggtggcgcccatcgtccagccggtggcggtcttggtcatggtgacctcgatctcgcgctccgtgccgatggagtcgtacgccttgaccgtgagggtcttgacggtgccctccttggcgtcggcctggaggttgccggcgaacggcgccgacgtcgtggccttggcgggcatgacggtgccgaccttgacgctgatgtcgccgatggcgccggaggtgtcgatgacgccgtcctgcgcggcccagccctgcacgatcgcgccgtcgcccggcaggaccatctggccggaggagtcgaagtcgaacgagccggcgcgcgtgtagtactgctgcgtgccctgacggaccacgaagaagccgtcgccggagatcatcatgtcggtgctgcggccggtgagctgggcggcgccctgcgtgaagttggtggtgatgccggc

SEQ ID NO: 48 - DNA, 478 bp, Enterobacter sp.
  misc_feature 1..478: note = Marker nucleic acid sequence
  source 1..478: mol_type = genomic DNA
cgacggcgaccagccgggacggcgggatgtcgagcgcgtgccgcacccgctccatcgccgtcgccttgctgatgccgtccggggagatgtcgagccacgccgtccagccgatcgagtagctcacccgctgcagacccatccgctcgacgatggcgaggaactcctcctcgtcgtgctgcggcgacaccaccacgacgcgggtcgccgggtgcactgcgagctcctcgcaggagacctgctcggcgttcaccagctcccagtcggtcatgccctcggtgtagcggcgggagccggtcgggtcctcgaccatgaaactgccggggggcagggggggccggatggtgtgcagcaccccgggcgggacgaacgtcccggttaactcccgccgggaaccgccctcaaccggttcgctgcgcatcatcgttaccccgccgtttgtgcccaccacgaatctggtggtcgcggctgaacttctctt

SEQ ID NO: 49 - DNA, 461 bp, Enterobacter sp.
  misc_feature 1..461: note = Marker nucleic acid sequence
  source 1..461: mol_type = genomic DNA
gtggatgttcagtgtgagccacggcgcgggcggctgcctcacaagcaccagggcatcgccccagcgatagatatcgcgaataaagacgtttttcttgttccccccgacgtgtgagcgattctcaccaaacgcgggcgcaacaaatatatccgcctgttcggaaaactcggttatccagtgctgatagttttcccgcggatagtggccccgcgcgcggtcaggcccgccatggtttttcttttcggcctgctcatcgcccaccacccccaggtcggttaacgtcgactcgccctcgactcaaattttggccgtggccatcgggccgctgccctagtacttccttaccttgcatgtaagtgccttcgccgtaaactgcaccaccatccctctcggcaagtacacatacagccgtcccgcacactcgctgctaaccggccgaacaccaaccgtattacttgaca

SEQ ID NO: 50 - DNA, 454 bp, Enterobacter sp.
  misc_feature 1..454: note = Marker nucleic acid sequence
  source 1..454: mol_type = genomic DNA
ggtagggggagcacagccccagacaacagaacccgacggcccaggccaagcacgcaaagcaagcgtatcatcccagtgcgcagggcataccggcagcacgcgtccccgcggggacacccccggcggggtggggttttgtttaaattcccaccggcccgcccccgccaggccgagcgaaaccggccccccaaaatgcggaagaaaaaaaaacgccggtttaataaaaaaaaaaagagggtgcgttttttcttgtaaatttgaatataaaaccgtgattccattaacagctgtttatattttttttttaacagcggtgttgaactattgcttcttaggagccccgccaacgataatgaacgaaacaggagtatcggaattgaaaaagcgatttttaacctactactaagttctttataacacttaaaacaaaatgtcacgaatgcaaaaacgaaca

SEQ ID NO: 51 - DNA, 437 bp, Enterobacter sp.
  misc_feature 1..437: note = Marker nucleic acid sequence
  source 1..437: mol_type = genomic DNA
tttgtttgtgttgtgggaaaaatctatgatcgcataaatatttgtggtctctcccttagtttgcgcccgtacccaccttctttgtgtttcctccacacccacttacgcggcggcccccccccgttgtttgttttcggcagcgtacttttttgcacccgcggggcgcgggggggtggtgggggtgggcgccccccgcccccccgtttttggggttttttaaatatttttttttttttttaaatgaaaacgttaaaggcggataatttttaaaggaatggttaacatcctggctttttcggagaagtattttaataatgatacgtgaacaaatagaaaataaattaagggcagcgttcaaccctgttttcctcaaagtcgtcgacaaaagctatcgtcataacgtcccggcaggttctgaaacccattttaaagtggtt

SEQ ID NO: 52 - DNA, 332 bp, Enterobacter sp.
  misc_feature 1..332: note = Marker nucleic acid sequence
  source 1..332: mol_type = genomic DNA
cgcgccagcagccggcattgcccgacgaggagcctgaactctctttcccgtaggcggctcagccgtttcgtccctcctcattcacgcgtttcagggccgcatcggcttttagcttcagctcatgcagcgtatcgccatcctgcgggtagaggctgacccccgcgctgattgttgtgctcaacgtgtgcccacaaagtgaaaacgggcggcgcatatcctccagcaatgtcgtgagcagcgcgatgagtttatcgtcgtcacactcgggaaccagcaggataaaggcgtcgtagccaagcacggggagggccatatggagggtgaggcgggtg

SEQ ID NO: 53 - DNA, 489 bp, Pseudomonas sp.
  misc_feature 1..489: note = Marker nucleic acid sequence
  source 1..489: mol_type = genomic DNA
gctcaccacctggtggtggacggtgtgtcgtggcgcatcctgctcgatgatctgcaacgtgtgtatgaacagttgcaggcgggccagacgccgacccttgggcacaagaccagtgcgttccagcgctggggcgaagtgctcctggagcaggcgcccgggcgcctggcggagctggagttctggcgcgctacggttgcggcaggggccgtcagcctgccgctgctggacgctgcgggcagccgccgtcgtgaccaggtgcgcgagtgtcaggtgcgcctggccgagcccctcacgcgtcagttgctgacccaggcgccgcaagcctatcgcagccgcgtcgatgaactgctgctcaccgcgctggcccgtgtggtcttgcgcgccactggcggtcagagtgtgctggtggccctggaaggtcatggtcgcgaggtcccggcgcaatacagcgatgtcgacctgagccgcagcgtcggctggttcaccagt

SEQ ID NO: 54 - DNA, 487 bp, Pseudomonas sp.
  misc_feature 1..487: note = Marker nucleic acid sequence
  source 1..487: mol_type = genomic DNA
tgcaggaacacgctggcccgggaggatttggccaggccgtcgaacgagaggggcggctcgtaccagcggccgttggaccagcactccaggtagtcgaggatgccgcgctcgtcgagcaccggtgtgggttcgccgaaggtgaacacctccatgcaagcggcgggtgctggcagctgttctggaatgtcgttcatcagtagatctccatgaacccggtgttggtggcggtctgcccctccagcggttcgttctgcagtgcgtggaaaagcgcccaggccaggtcggcgtggccggtctcgtcggtgcggccggcggtgtaggtgaactggcggccgctggcggtgacggtcttgcggatggccatgagcgactgggccatgtcgatccagccggcgtcgaattccagccggcctttgtgaatgacgtcgtaggccttgagcaccaggcgggttttcacttcgggcgagtagctgaaggtggtcaggtt

SEQ ID NO: 55 - DNA, 484 bp, Pseudomonas sp.
  misc_feature 1..484: note = Marker nucleic acid sequence
  source 1..484: mol_type = genomic DNA
gacgtactccagccggcaatcgatgccgtcagggttggcaatgacatcgagggtgaggtcgaaacgcgcactctccagctccacgtccaacacctgcacctgcaatcccggcagttgcagcgcctgggcatcccgcgaatggcgaaagttgaacagtacctggaacagcgccgtgtgatgcagatcgcggctcaggttcaggccgtccatgacgcactcgaagggaaaatccgattgctccagcgcgacacggctttgctcgcgcaaacggcagcacagcgcgcgcgtggtcagcgcaggctccagccgtgcgcggtacacctgggtgttgacgaagaaaccaacgatgttctgcacctgggcatgactgcgcgcagcgttgggcacaccgacggcaaagtcgcgctggccgctgtagcgggccaacagcacttgccaggcgcccagtaacaccacgaagggcgagcactgctgcgatcggcag

SEQ ID NO: 56 - DNA, 477 bp, Pseudomonas sp.
  misc_feature 1..477: note = Marker nucleic acid sequence
  source 1..477: mol_type = genomic DNA
taatctgcaagtggacagcctgtggaccggcgccttgcatctggtcgcagtggaactggacaggccgcagactcaagtactgttcgacaaaagcggcaaactgaacctgagcgctctgttcaagcttccggccagcgataccgctgccgagcaggacgcgccttccgagcccttcgccttgcgcatcggcagcatcaagctggtcgatgggcgtttgcatttcaaggatctgcgccccagccagcccatcgaatttctatacgactcgatgaatctggagctgcagaacctcagcacattgccggacgatcatgccgacatgaccctggttgccaacagccctcagggcggtcgtatcgactggcgcggccggatcggcctgagtccggtgtcgtcccaggggtcgttgaaggtgaccgatgcgcagatgagcgtctggtggccgtacgtgcgcgacagcgtgccgttggttctgga

SEQ ID NO: 57 - DNA, 472 bp, Pseudomonas sp.
  misc_feature 1..472: note = Marker nucleic acid sequence
  source 1..472: mol_type = genomic DNA
ctgccggcactgcgcgaagccatcgccggcttctatcgacagcgctatggcctggacattgatccccagcgcatcatgatcaccccgggcggctcgggcgccttgctgctggcggccagcctgctggtcgatcccggcaagcactggcttctggccgaccccggctacccgtgcaatcggcacttcctgcgcctggtcgaaggcgctgcccaactggtcccggtgggtcctgcacagcgctaccaactcaacgcccaactggtggcgcagcactgggacgagcacagcgtcggagccttggtggcgtccccggccaaccccaccggcacgttactgaatcgcgacgaattgcgtgccttgagccaggccgtgaagggccgccagggccatcttgtggtcgacgagatattgcaatcaacggccacacgccggatttcgcttccagcgccatgctgccgcccgaaggcctcga

SEQ ID NO: 58 - DNA, 374 bp, Pseudomonas sp.
  misc_feature 1..374: note = Marker nucleic acid sequence
  source 1..374: mol_type = genomic DNA
ggcggtctgttcccgttcctgttcatcaccatcgcctgcggcgcggtttcggggttccatgcgctgatctcctcgggcaccacgcccaagctgctggataacgaaaccaacgcccgctacatcggttacggcggcatgctgatggagtccttcgtggcgatcatggccatggtggccgcttcggtgatcgagccgggcgtgtacttcgccatgaacagcccggcggcgatcgtcggtaccgatgtggtggccgtggcccagaccgttagcagctggggctttgcaatcacccccgacgcgctgcaagcggtggccaaggacatcggcgagaccaccatcctggcccgtgccggcggtgcgccgaccctggcggt

SEQ ID NO: 59 - DNA, 212 bp, Pseudomonas sp.
  misc_feature 1..212: note = Marker nucleic acid sequence
  source 1..212: mol_type = genomic DNA
accgccagggtcggcgcaccgccggcacgggccaggatggtggtctcgccgatgtccttggccaccgcttgcagcgcatcgggggtgattgcaaagccccaagtgctgacagtctgggccacggccaccacatcagtaccgacgatcgccgccgggctgttcatggcgaagtacacgcccggctcgatcaccgaagcggccaccatggccat

SEQ ID NO: 60 - DNA, 634 bp, Pseudomonas sp.
  misc_feature 1..634: note = Marker nucleic acid sequence
  source 1..634: mol_type = genomic DNA
cctacgaaaccatcgacgtcaccctgaaggacacctcggcgactgccctgggttccaatcaggttggtagcagttctggtaccgctgccggtaccactgccggtaccgtggttgccggtagcggcaatgccttgacctctagcggcactattaccctggtgggcggtggcaagaagcaggacgtgacctatgctgcaggcgactccgccaagaccatcgcagcgggcatgaatggtcagatcccgggcctcgccgcctctgcgcgtaccgtcctgaccgtgaccgacaccatctccagcggcgcggccaacatgaccatgaacgttggcagcaactcgctgaacctggtgggtgtgaccagcaccaaggacatggccgaccagatcaacgccaacgccgccaagcttggcgtcaccgccaactatgatagccaatccaagaagctgactatcacctcggcgaccggtgagaacatcaccttcggcaaggacacgggcaacgcggcaggcaacatcaatgtggcctcgcagaggtccgatggtaccttcagctccgcggtcgatgtccgcgccaacggtggccagggcatgggctatgtcaagttggattcgccgacgaccttcgccatgaccgg

SEQ ID NO: 61 - DNA, 241 bp, Pseudomonas sp.
  misc_feature 1..241: note = Marker nucleic acid sequence
  source 1..241: mol_type = genomic DNA
cctgccaaatgccacagcgtgaagtgtccaccctgtctccgaacaggtgttcaccatgtccccgggccatacaggagggagagggggcgatcgagtccggggcgcgttacggttcagtcggtaggaggtatcgtctgatcgcggccatggcggtccgccgatgcggccgcttgtgtcttggcttgcggttaggatgaaggtgagagcagcagggggcaggctgtagggccgcagtgtttcg

SEQ ID NO: 62 - DNA, 413 bp, Gluconobacter sp.
  misc_feature 1..413: note = Marker nucleic acid sequence
  source 1..413: mol_type = genomic DNA
agcttgaatggactatggctcaatgcggcgttcgcagcacttgggacacctgaagaactagacgcattgaaattcgataatatgatggcgacgaatgtgcgggggccaatgcttcaactggcacggctctcgccaagtctggctccgggagcatcagtcgttgtaacgtcctcaagttcgacctatgagggtgcagcggtcactggcctctatgctgcaacaaaaggtgctgtcgttgccatggcacgctcttgggctacagctttggctccacgtggcattcgcgtaaatgtccttgtcccaggcccaatcgagacaaatttccgcagttttttgccagatgaagcgcggaagggatttgaggacttcgtgcttaatcaagtccccctcaaacgggcaggaacgcctgaaga

SEQ ID NO: 63 - DNA, 396 bp, Gluconobacter sp.
  misc_feature 1..396: note = Marker nucleic acid sequence
  source 1..396: mol_type = genomic DNA
atggcctggagcttcatgatgatggcatcactgcctatcattcatggtggtcgctatacggcggagattgcccaggcgcgtgcggaagcagaagccagccggctgacgtatcgcaagacagtgctcaaggcgtttgaggaagtcgaagactctctcggtgactggcggcacgataatgaactggtcagccagctcgaagatgcagcccgggactccggactggctcgtgatcgggcgcagaagctgtttggtgcaggtctgacgggctatctgaatgttctgaccacggagcagacagccctgaccgcacaggatcaggctgttgttggccgtacggcccgcctgcgggatgctatttcgctctacacggaaatgggcgctggctggcagggacgt

SEQ ID NO: 64 - DNA, 330 bp, Gluconobacter sp.
  misc_feature 1..330: note = Marker nucleic acid sequence
  source 1..330: mol_type = genomic DNA
cctgtagatttgacgatttcggcaagtgcttctgccgtgggatcagcagagtcatttcttacgacgatggctcgatccccaaattcctctttagccgatcgcaatctgtcttcgctcagacccgtcagaatgacttggccgccttccaagatgactcgccgtgctccggcaagtcccatgccacttgtcccacccgtgattaaaatgcgctttccatcaaatcttgccattaatccgacctccttttttataaaaacattctcacacaacgtgtgtccgttttgcgacatcagtgacgtgtttttgctaatgcctaaatcacgagcgatc

SEQ ID NO: 65 - DNA, 289 bp, Gluconobacter sp.
  misc_feature 1..289: note = Marker nucleic acid sequence
  source 1..289: mol_type = genomic DNA
gggcgcatcccgccagcgcatcccattgcggttcacgaaaatgatgccgctcagcacgcgacggtcatcaacgcgggctctaccatggctctttgggaaaaagggctgcagacgcttcatttgttcgtccgtcagccaaaacaggtcgctcattgccagtctcctcacagagcctgaatcagatttccataatcaaatcaatgggtcctgagcctaacactacagttgtattttgatgtgatatctgattctttgtcctgtgatggaacaggatatgatgacaggcgga

SEQ ID NO: 66 - DNA, 267 bp, Gluconobacter sp.
  misc_feature 1..267: note = Marker nucleic acid sequence
  source 1..267: mol_type = genomic DNA
aaacattctcacacaacgtgtgtccgttttgcgacatcagtgacgtgtttttgctaatgcctaaatcacgagcgatccactggtagcttgcggcctttagaagctggcgctttgtcccagagaaagtccccggaaaaggcgctgtacccccatcctaccggggaagtatgcgccagaaaatcgttagggacggccgccgatgtcgaacgcagatgcgaaatagcggcttgcagatagacagcgttccagtagacgatcgccgcaata

SEQ ID NO: 67 - DNA, 639 bp, Bacillus sp.
  misc_feature 1..639: note = Marker nucleic acid sequence
  source 1..639: mol_type = genomic DNA
tttttttccaaggacaagaggaagaataataccgaaattttttatttaggaggtgtagaccttacacacgtaaggtttgccattggataatataaccgttaactttatactagttgccatcttaattgcattcacagcatttttcgtagcaacagaatttgccattgttaaagtcagaacttctagaattgatcaactggtcgctgaaggaaaaagaggagccattgcagctaagaatgttacaacgcaccttgatgaatacctttcagcgtgtcaattaggaattaccgttacagctatgggactaggttggttaggggaaccaacgatcgaaaaagtattgcatcctttatttgcagcattagaactgaatgaagcgacaactactattctatcgtttggtattgcttttgctattatgacctatctccacgtcgtaattggagaattagctcctaagacgctagccattcaaaaagcagaatggattacgttaacgctcgcaaaaccaattatttggttttatcgcattatgttcccttttatttggttattaaatgggtcagcccgtcttgttgtaggaatatttggcctaaaaccggcctctgaacatgaaatggcacactctgaagaagaatt

SEQ ID NO: 68 - DNA, 606 bp, Bacillus sp.
  misc_feature 1..606: note = Marker nucleic acid sequence
  source 1..606: mol_type = genomic DNA
tattcgtggagcaatatatgattgccaagccatatagtattcgataggtatttgctccaataattcctctttatttgcaaagtgataggaaataacccccttactgatatttgcacgttttgcaatccgtcctaaagaagcttgagcgtaacctacttctgcgattgtttcaattgcacattccacaatttgagctctacgggctttttcgatgaatgacagttgtttttggctagtcggcttattttttttatttatgttcttattttagtacattcgtacaaataattcaaacaaaaaaaccatttaggtgaagattacctaaacggtttttaaacctctttatacaaatgaaaagaatccatttcgatcaaaatggattcttttccaataattacctgtccactccacaaaaagtgaatacaatcatatcgttcgcaaagtgtacgtccgtaaaagtttacttttacggccatttctttttgattagaaatctagtatttttcgtgttcatttaagctggaaatcaaattacgaacgtccttaaaaatacatacacttttacggacgtttttgatagaataatagggagagaaacacaaaagg

SEQ ID NO: 69 - DNA, 523 bp, Bacillus sp.
  misc_feature 1..523: note = Marker nucleic acid sequence
  source 1..523: mol_type = genomic DNA
aatttctcctcgggatattttcatcgataagcaaagtggaaaaaacttcaatcgagaacagtatcaactgatgaaacgaatgatgcgtaaaggggatattctttatattcattctctagatcgcttcggacgtaataaggaagaaattttacaagaatggaatgccattacaaaagagattgaggcagacattgtagtcttagatatgccgttgttggataccactcaatacaaggatagtttgggaacctttattgcagatttagttttgcagattctttcgtggatggcagaagaggaacgagatcgtattcggaagcgtcagcgtgaaggcattgatgctgcactaaagggtggaatctcttttggacggcctaaagctcaggttagccaagaatttattgaagcttataaccggtggagaaataaggagattacagctgtacaagccatgaaagaggccaatgttaaaaagacaaccttttataaattggtgaaggaatatgagggtacttttaataag

SEQ ID NO: 70 - DNA, 446 bp, Bacillus sp.
  misc_feature 1..446: note = Marker nucleic acid sequence
  source 1..446: mol_type = genomic DNA
tcagcccgtcttgttgtaggaatatttggcctaaaaccggcctctgaacatgaaatggcacactctgaagaagaattgcgtctcttactttcagagagttataaaagtggagaaattaataaaaatgaattgaaatatgtaaataatatttttgaatttgacgagagaattgccaaagagattatggttccgcgaacagaaatggtaacgttggatgcgggggactcattcaaccaggctatagagatattaaggaatgagaaattcactcgttatcctgtcgtagatggagataaggataatattgttggggttgttaatatcaaagaaattctaaccactacgttgtgggaaaaggatgagaaagcaaaccttagggattttactcatcctgttattcaagttattgaaacaatacctgttcatgaattaatgattaaaatgca

SEQ ID NO: 71 - DNA, 245 bp, Bacillus sp.
  misc_feature 1..245: note = Marker nucleic acid sequence
  source 1..245: mol_type = genomic DNA
ggtccaagatcaccagtagcacccgtaggtccagttaatccaagatcaccagtagcacccgtaggtccagtcggtccgatatcgccagtagcacccgtaggtccagttaatccaagatcaccagtagcacctgtaggtccagtcggtccgatatcgccagtggcccccgtaggtccagttggtccaagatcaccagtagcacctgtaggtccagttggtccaagatcaccagtagcacccgtagg

SEQ ID NO: 72 - DNA, 306 bp, Pseudomonas sp.
  misc_feature 1..306: note = Marker nucleic acid sequence
  source 1..306: mol_type = genomic DNA
cattatcgatactcaaagtaccgggaacgactggaaagagagggcgtggagcagagcatgtcacgccgaggaaactgctatgacaatgccacaatggagagtttctttggcacgttgaagtcagagttttattatcgggaacgcttcgatagcgtggcccagttgcaagccggactcgataaatacatccattactacaatcatagacgaatcaaaaccaagcttggcggactgagccctgtagaatacagagcccggtccgctaagacctagacaataactgtccagcttttggggcgcacttca

SEQ ID NO: 73 - DNA, 20 bp, synthetic construct
  misc_feature 12: note = n is a, c, g, or t
  misc_feature 1..20: note = Primer
  source 1..20: mol_type = other DNA
agagtttgatcntggctcag

SEQ ID NO: 74 - DNA, 22 bp, synthetic construct
  misc_feature 6: note = n is a, c, g, or t
  misc_feature 1..22: note = Primer
  source 1..22: mol_type = other DNA
tacggntaccttgttacgactt

SEQ ID NO: 75 - DNA, 19 bp, synthetic construct
  misc_feature 9: note = n is a, c, g, or t
  misc_feature 1..19: note = Primer
  source 1..19: mol_type = other DNA
gtgccagcngccgcggtaa

SEQ ID NO: 76 - DNA, 20 bp, synthetic construct
  misc_feature 11: note = n is a, c, g, or t
  misc_feature 15: note = n is a, c, g, or t
  misc_feature 1..20: note = Primer
  source 1..20: mol_type = other DNA
ccgtcaattcntttnagttt